European Patent Specification EP 4 048 680 B1, published January 31, 2024. Title: PEPTIDES WITH PROTECTIVE ACTIVITY FROM CELL DAMAGE AND LIPOSOMIAL FORMULATIONS. Applicant: I.R.A. ISTITUTO RICERCHE APPLICATE S.P.A. The sequence listing filed with the application follows.

SEQUENCE LISTING (8 sequences)

SEQ ID NO: 1 - protein, 12 aa, Artificial Sequence
  NON_STD 1: if present is, CF (carboxyfluoroscein), palmitoyl (CH3(CH2)14CO-), oleyl (CH3(CH2)7(CH)2(CH2)7 CO-), stearyl (CH3(CH2)16CO-), lynoleil (CH3(CH2)4(CH)2CH2(CH)2(CH2)7CO-), or lynolenil (CH3CH2(CH)2CH2(CH)2CH2(CH)2(CH2)7CO-)
  SEQ ID NO:1
  NON_STD 2: if present, is Aib
  NON_STD 3: Trp, Phe or Tyr
  NON_STD 4: Trp, Phe or Tyr
  NON_STD 5: Lys
  NON_STD 6: Tyr, Trp, or Phe
  NON_STD 7: Tyr, Trp, or Phe
  NON_STD 8: Gly or Ala
  NON_STD 9: Lys
  NON_STD 10: Ala, or Aib
  NON_STD 11: Ile, Leu or Ala
  NON_STD 12: Tyr
XXXXXXXXXXXX

SEQ ID NO: 2 - protein, 11 aa, Artificial Sequence
  NON_STD 1: Aib
  SEQ ID NO:2
XWFKYYGKAIY

SEQ ID NO: 3 - protein, 10 aa, Artificial Sequence
  SEQ ID NO:3
WFKYYGKAIY

SEQ ID NO: 4 - protein, 11 aa, Artificial Sequence
  NON_STD 1: CF (Carboxyfluorescein)
  SEQ ID NO:4
XWFKYYGKAIY

SEQ ID NO: 5 - protein, 11 aa, Artificial Sequence
  NON_STD 1: palmitoyl (CH3(CH2)14CO-)
  SEQ ID NO:5
XWFKYYGKAIY

SEQ ID NO: 6 - protein, 10 aa, Artificial Sequence
  SEQ ID NO:6
  NON_STD 8: Aib
WFKYYGKXIY

SEQ ID NO: 7 - protein, 11 aa, Artificial Sequence
  NON_STD 1: palmitoyl (CH3(CH2)14CO-)
  SEQ ID NO:7
  NON_STD 9: Aib
XWFKYYGKXIY

SEQ ID NO: 8 - protein, 11 aa, Artificial Sequence
  NON_STD 1: CF (Carboxyfluorescein)
  SEQ ID NO:8
  NON_STD 9: Aib
XWFKYYGKXIY